European Patent Application EP 4 129 335 A1, published February 8, 2023. Title: ANTI-C-MET ANTIBODY-DRUG CONJUGATE AND APPLICATIONS THEREOF. Applicant: REMEGEN CO., LTD. The sequence listing filed with the application follows.

SEQUENCE LISTING (10 sequences)

SEQ ID NO: 1 - protein, 5 aa, Artificial Sequence
SYWMH

SEQ ID NO: 2 - protein, 17 aa, Artificial Sequence
MIDPSDSESRLNQKFKD

SEQ ID NO: 3 - protein, 13 aa, Artificial Sequence
SGYHGTSYWYFDV

SEQ ID NO: 4 - protein, 16 aa, Artificial Sequence
RSSKSLLHSDGITYLY

SEQ ID NO: 5 - protein, 7 aa, Artificial Sequence
QMSNLAS

SEQ ID NO: 6 - protein, 9 aa, Artificial Sequence
AQNLELPPT

SEQ ID NO: 7 - protein, 122 aa, Artificial Sequence
QVQLEQSGPEVVKPGASVKVSCKASGYSFTSYWMHWVRQAPGQGLEWMGMIDPSDSESRLNQKFKDRVTMTVDTPTSTVYMELSSPRSEDTAVYYCARSGYHGTSYWYFDVWGQGTLVTVSS

SEQ ID NO: 8 - protein, 115 aa, Artificial Sequence
DIVMTQSPLSLPVTPGEPASISCRSSKSLLHSDGITYLYWYLQKPGQSPQLLIYQMSNLASGVPDRFSGSGSGTDFTLKISRVEAEDVGVYYCAQNLELPPTFGGGTKVEIKRTV

SEQ ID NO: 9 - protein, 452 aa, Artificial Sequence
QVQLEQSGPEVVKPGASVKVSCKASGYSFTSYWMHWVRQAPGQGLEWMGMIDPSDSESRLNQKFKDRVTMTVDTPTSTVYMELSSPRSEDTAVYYCARSGYHGTSYWYFDVWGQGTLVTVSSASTKGPSVFPLAPSSKSTSGGTAALGCLVKDYFPEPVTVSWNSGALTSGVHTFPAVLQSSGLYSLSSVVTVPSSSLGTQTYICNVNHKPSNTKVDKKVEPKSCDKTHTCPPCPAPELLGGPSVFLFPPKPKDTLMISRTPEVTCVVVDVSHEDPEVKFNWYVDGVEVHNAKTKPREEQYNSTYRVVSVLTVLHQDWLNGKEYKCKVSNKALPAPIEKTISKAKGQPREPQVYTLPPSREEMTKNQVSLTCLVKGFYPSDIAVEWESNGQPENNYKTTPPVLDSDGSFFLYSKLTVDKSRWQQGNVFSCSVMHEALHNHYTQKSLSLSPGK

SEQ ID NO: 10 - protein, 219 aa, Artificial Sequence
DIVMTQSPLSLPVTPGEPASISCRSSKSLLHSDGITYLYWYLQKPGQSPQLLIYQMSNLASGVPDRFSGSGSGTDFTLKISRVEAEDVGVYYCAQNLELPPTFGGGTKVEIKRTVAAPSVFIFPPSDEQLKSGTASVVCLLNNFYPREAKVQWKVDNALQSGNSQESVTEQDSKDSTYSLSSTLTLSKADYEKHKVYACEVTHQGLSSPVTKSFNRGEC